European Patent Application EP 4 428 242 A1, published September 11, 2024. Title: Method for determining risk of adverse event. Applicant: 株式会社ヤクルト本社. The sequence listing filed with the application follows.

SEQUENCE LISTING (4 sequences)

SEQ ID NO: 1 - DNA, 78 bp, synthetic construct
  source 1..78: mol_type = other DNA
aatgatacggcgaccaccgagatctacactctttccctacacgacgctcttccgatctagrgttygatymtggctcag

SEQ ID NO: 2 - DNA, 88 bp, synthetic construct
  source 1..88: mol_type = other DNA
caagcagaagacggcatacgagatnnnnnnnnnnnngtgactggagttcagacgtgtgctcttccgatctgctgccwcccgtaggwgt

SEQ ID NO: 3 - DNA, 21 bp, synthetic construct
  source 1..21: mol_type = other DNA
cggaactgaagatttggtgat

SEQ ID NO: 4 - DNA, 21 bp, synthetic construct
  source 1..21: mol_type = other DNA
gtaccaccggagtttttaccc